European Patent Application EP 4 700 134 A1, published February 25, 2026. Title: 신규 우결핵 바이오마커 및 이의 용도. Applicant: 주식회사 제노헬릭스. Application KR. The sequence listing filed with the application follows.

SEQUENCE LISTING (35 sequences)

SEQ ID NO: 1 - DNA, 3977 bp, Bovine
  source 1..3977: mol_type = genomic DNA
gataaggaccttctcagcagcgctggagttttcctggttacctgccggataagctctccagccctccaactcaccatgtggtgagttcaaggtccagtccaacagcacaggggaattcacactagccctgagccctgaagatggtgtcacagtcttcgggccggcaggactcacctgtggacccctgggaaggggtcagcgatgacccaggcaacactgatggcttgcccagcctcctggacactgagcaccccttctgcccctcagacatcaggttcacaaggcacagagctgcctggattaaccctccgtgtgcgcagcaacagctgcaggatgcatccccccaggtgctcgcagtggggaacagagagagccacactgcgtccaacaccaaatctcccttgggcacttcacccttgtctcttggtgactccgtggtggagacatcactgccgaagggcaccacagactctctgggcagctcctctgcctggggcacagctggcaatggcagtgactcctctgttaccttgaaggaagagcgggcagggcttccaagacgctgtcctcacacatctctgatcacgagctccaagactgtgtctggtcccccatgtcctgaggatggcagggcttttttcaagccttcccagctgacagcttctgctgatgcagatgctgttcaagttggcggaagaactgtttcctcaaattccttctcaccggaggcattcgttcttcctgttgatgcagaaaaggaaaatgcccacttttacgttgcagatatgattatatcagtcatggagaaaatgaagtgtaatattctaagtcagcagcacacagagacctggagtacagaagaggccggcaggtcacttgggaacagtcgggcagacttggaagggaccttttatacccacgtaaagcaggaatctgggtcttccacttcgtctgacagtggctatgaaggttgcgtgttacaggtcagcccggtggttgaaacacctactttctctgaggtgacggaagaggactgcaaatgtgactttgatgacttcgttatcgtagaacttggagatttcagcaataccacagagccctgtggatgttcctccgacacctctaagagtgtcattcatgagccaaacttcaattctgctgagctaatagccaaagagttataccgcgtattcaggaaatgctggatgctggcagaagttcattatcagctgacaggctctctcgatgcagctggctccatagttataaatgaagagcgggttcagaaagactttgaatccagcacagatgttgtccaggaaattaaactgaagtcgaggatcagagggactggagactgggcgccccctaggtttcaaatcatatttgatattcatccaccactcaagagggatctcgtggtaatagcccaaaattttttctgtgctggctgtggaactccaatagaacctaagttcgtgaagcggctccggtactgcgaatacctggggaagtacttctgcgactgctgccactcctactcggagtcctgcattcccgcccggatcctcaggatgtgggacttccggaagtactacgtcagcaacttctccaaacgcctgctggaccacatatggcacgagcccatcttcaacctgctgcacgtcagccacggcctgtacaccaaggccaaggaactggacagagtgagggaaatccaggagcagctgtttcatatcaagaagctgttgaagacctgcaggtttgctgaaagcacattaaaggagtttgagcagctgccaggacacttgacggaggcgctccacttgttctccctggaggacatggtcaaggtcaagaaagggctgctggcgcccttgctcaaggacattctgaaagcttccctcgagcacgtggccagctgtgagctatgtcaaggaaagggcttcatttgtgaattttgccggagtacagctgtcattttcccatttcagactgcaacgtgtagaagatgttcagcgtgcagagcttgctttcacaagcagtgcttccagtcctccaagtgcccccggtgtgcgaggatcacagcgaggagaagacttctggaaagtctaccctccgcagcaacatgatgtacttgactgtatcgagaaagaccatgcaacatgccttacgatcacatcgcttgtgtctcctgttgataacattgtttgactattgtctattactcctgttgataacattgtttgactattgtctattaagaaaaaagatgaccaatattctctttattatatatatttaatatttttggaaacttcggatctttgttattaagagtagagttgttactggtgccaaagaatgctcaaactaccgcacaattgcactcatctcacatgctagtgaagtaatgctcagaattctccaagccaggcttcagcaatatgtaaatcatggaccatgaatgtttcaagcatggaccagatgtttaagctggttttagaaaaggcagaggaaccagagatcaaattgccaacatctgttggattgttgaaaaagcaagagagttccagaaaaacatctatttctgctttattgactatgccaaagccttggactgtgtggatcacaataaactgtggaaaattctgaaagagatgggaatcccagacctcctgacctgcctcctgagaaatctgtatgcaggtcaggaagcaacagttagaactggacatggaacaacagactgggtccaaatagaaaaaggagtaagtaggtcaaggctgtatattgtcaccctgcttatttaacttatatgcagagtacatcatgagaaacgctgggctggatgaagtgcaagctggaatcaagattgacgggagaaatatcataacctcagatatgcagatgacaccatccttatggcagaaagtgaagaactaaagagcctcttgatgaaagtgaaagtggagagtgaaaagttggcttaaagctcaacattcagaaaacgaagatcatggcatctggtcccatcacttcatggcaaatagatggggaaacagtggctgactttatttttctgggctccaaaatcactgcagatggtgattgcagccatgaaattaaaagatgcttactccttggaaggaaagttatgaccaacctggacagcatattgaaaagcagagacgttactgtgtcaacaaaggtctgtctagtcaagacagactatgccaaagccaaagccaaaaagactatggcttttccagtggtcatgtatggatgtgagagttggactataaagaaagctgagcgctgaagaattgatgcttttgaactgtggtgttggagaagactcttgagagtcccttggactgcaaggagatccaaccagtccatcctaaaggaaatcagtcctgaatattcattggaaggactgatactgaagctgaaactccaattactttggctgcctgatgcgaagagctgactcatttgaaaagaccctgatgctgggaaagattgagggcaggagaaggggatgacagaggataagatggttggatggcatcaccgactcaatggacatgggtttgggtggactccaggagttggtaatggacagggaggcctgctgtgctgtggttcatggggttgcaaagagtcgaacacaactgagcgactgaactgacctgaactgttactggtgattttgtttacaaatgttcgatgtttttgctgctactggtgttttttttaagggttttttgatacttcttaaattgtatttaaatggttgtatttagctaatggtggagcctgttttttatgaattataactgacaaggtgaattactcagttcctattcctataaagcttgttttgtgaaaggaattgttactttcaatgaacaaaaactgaaaacaaaaaaaaaaaaaaaaaaaaaaaaaaaaaaagaaaaaaaaaaaaaaaa

SEQ ID NO: 2 - DNA, 1091 bp, Bovine
  source 1..1091: mol_type = genomic DNA
ctcagccagcgctcccgccagccttcccgcagcagacacagaccctccgagctgagactcatggccccagccgcgaccgccgccgccccccggctcctccgcgcagcgatgctgctcctgctcctggtggccgccggccggcgcgcagcaggggcgcccgtggtcaacgaactgcgctgccagtgcctgcagaccttgcaggggattcacctcaagaacatccagagcgtgaaggtgacaacccccggcccccactgcgaccaaaccgaagtcatagccagtctcaagactggtcaggaagtgtgtctcaaccccaccgcccccatggttaagaaaatcatcgataagatgctaaacaaggctagtgccaactgatcaagagagatggaacgagcttcttgatactccagcagcctcagtggaagtgaagtaaaagaagagaaacaaatggttcccggggccatctggactgtgtttaatgtattttgctgtgtcttatgagagttctatttatttacatctgtatttatttatttatgtttcaaagcctgtgtattgatattctaatatttaaaggtgtgaatgtgtttggcagttcttggtactgttcgtttcaaagtttatttttatgttaacttatagttagttcaatcctgactgttatttaatttgaagatggtgtgttttaagtgttcttcacttattaaactatttttggggagagggtattccacactgtactatccactatagtaaaggctagagacagtagtggagggttcaagcaaacagataggtcacgatcactgttaatgtagggaatgtatgtatacatttactttttgtagagaagattgtcagttgttatttattgaaacatttcactgtctgtagtcaacatttctgatgttgaacctttacaaatgacaatgatctaaatatcccttggacattttatgtcttccttgtaaggcataatgccttgtttagtgtgagttatctaaatgtttctctatgtcttggaatagagaagtttaagtatttattgatgtatttttattaataacatgaaaataaagtttttacacaaa

SEQ ID NO: 3 - DNA, 1113 bp, Bovine
  source 1..1113: mol_type = genomic DNA
cgctcagccagcgctcccgccagccttcccgccgcctcagacacagaccctccgagcagacacccatggccccagccgcgagctccgccccccggctcctccgcgcagcaatgctgctcctgctcctggtggccgccggccggcgcgcagcaggggcgcccgtggtcaacgaactgcgctgccagtgcctgcagaccttgcaggggattcacctcaagaacatccagagcgtgaaggtgacaacccccggcccccactgcgaccaaaccgaagtcatagccactctcaagactggtcaggaagtgtgtctcaaccccgccgctcccatggttaagaaaatcatcgataagatgctaaactaggccagctctaactgaccaggtggaaaacagaagctcttggatggctgttccagaagtagaccctgcccctacagaaatcaaagagggaaaagaggaatcaccacctcctaaggccatctggatcaggcttaatatgtttgaacatctcttaggagggttcttccacttatttacttatttatttatttatgtgttgcttgggtttcaaagattctatgttaatatttacatgtgacatgattaaggatgtgatcaaatctacttgcacatcctgtcattattggtattatttattttatgagaaaaaaagtttatttagtcctgattcttactgagtttgaagtagaaggtttgcaaatgtttgccagtcatgaaattaatatttctgaggagcccacattatgccagcccttgtggcagaagctggaggatcgaaacagatagtgaactcattgtcgggtggggggatacatgtttttgtgaatgtttttgtaaatgcatgtgtttgtaaatgtttaaaagaatgttagttatttattgaaatgatttcacagtatgttgtcagcatttctcatgttgaaactttaagagctacaatgttctaaataccctttggacattttatgtctttcttgtaaggcacaatgccttgtttcatgttaattatgcagtgcttttctatgtctgagaaaagagaaatctaaatatttattgatgtttttacaaagaacatgaaaataaaatatttcaa

SEQ ID NO: 4 - DNA, 1368 bp, Bovine
  source 1..1368: mol_type = genomic DNA
cgaggtttccgcttcctgttctgacggacgctccggccgtaacgatgatcggggacatcctgctgtttgggacgctgctgatgaacgccggggcggtgctcaactttaagctgaaaaagaaggacacgcagggctttggggaggagtcgagggagcccagcacaggtgacaacatccgggagttcctgctgagcctcagatactttcgaatcttcatcgccctgtggaatgtcttcatgatgttctgcatgatcgtgctgtttggttcctgagctccagatgcagaaccgagaacacaccttctgagtctctcttgctccgttcctgacgacttcaagaatgtttctgaccagaaaccgactgaccttcccagaaagtccaagcttgtggtgggtggaaaagatgttcgccaagatgctcatggtttcccagccacatcgctgttttctttacaaagatgttttctttgatcgctgccttgaaatgctgtctacttaaggagtctgaggagagtgtatgtaaagggctgggataatgttgcattccccaaagataaaagaacctatttaatcagagcagaatctctcttctaccaggctttccctggaaacctgtttctgtgtctttcttggtttattttcaataaccatccttttttggttcgagttatacggatttgtaaaaatctttcttaccagggatctgaagcagaaaggttcgcttttcggtttgatgcagcctcttattggactgtgtttgtgatgactgagcaagttcattgttgctgggtcagtgtccagattccttccccatcacaatggtttgtgctcgacgtactcagccacatggtaccactaaggttgccccaggacttcaagggtgaagtattattggttcccatggaagagaggtgcagagcagttggcagggtggatgggggttttatgagaaactttcccttgcctggaagccctctattaaagtaacttttggggaccattaattgtagagtttttagaatgagagtgatttatgtggtggtactgggatccagttctgaaagcttggtttcgggggtctgctttttaagtggatgatatcaagattgacaaactataagcctcatttgaggaaatacagcattttgcacagaagcttctttgaatccgagtccgaattttatcatcaacatggctgtctggtggtcagcacctggatcctgcaggtgtttgatttatttgttgtgatgtgtgaaatccaagcttctaggtaacctggtgggaggaaaaaataaatatgcaggcttttagaactaagtaggattgaaaataaagctcatttctaaaaagggcaaaaaaaaaaaaaaaa

SEQ ID NO: 5 - DNA, 1493 bp, Bovine
  source 1..1493: mol_type = genomic DNA
catcatggcaccaactgtccatctctcctgcctcctggccctgctggtggcaggcctggctcaaggcatcaaggactccctcaggggccaggacccaggtccccagccactggagctgaaagaggtcttcagattgtttcagatgcagtacaaccggagttatccaaatccagcagagtacgcccgccgcctggacatctttgcccaaaacctggccaaggctcagcggctgcaggaggaggacctgggcacagccgagtttggggtgactcaattcagtgacctcacagaggaggagtttgtccagctttatggaagccaggtggctggagaggccctcggtgtgagcagaaaagtggggtctgaagagtggggggaatcagagccccagacctgtgactggcggaaagttggcaccatctcacccgtcagggaccagcgaaactgcaactgttgctgggccatggcggcagcgggcaacatcgaggccctatgggccatcaagttcagacacttcgtggaggtctccgtgcagcagctgcttgactgtgaccgctgtgggaacggctgcaggggtggcttcgtctgggatgcgttcctcactgtcctcaacaacagcggcctggccagtgagaaggactatccattcaatgggagtggcaaaacccacaggtgcctggctaagaagtacaagaaggtggcctggatccaggatttcataatactgcaggcctgcgagcagagtgcgggcacaatggggacacgggtgggcacaggggggagacggacagggacagacggaccaggacagacggggctatagacagagacggaggccatctctgggggcgggggctagagggtggaaaagagcaagagatagatagagatgcccatgagccgagagcaggggatgaaggagtgacagggctagatggcaccttccacccccaggcatggccaggcacttggccaccgagggccccatcaccgtgaccatcaatatgacgctactgcagcaataccagaagggtgtgatcaaggccacacctaccacctgtgaccccacacaagtggatcattctgtcctgctggtgggttttggtaaaaccaagttggtggaggggaggcaggggaaggcggcctcgttcggatcccacgcacgccctcgccgctccatggcatactggatcctgaagaactcctgggggcctcagtggggtgaggagggctatttccggctgcatcgagggagtaacacctgcggcatcaccaagttcccggtcaccgccagagtggacaagcctaagaagcagcaccaagtctcttgccctccctgaggctgcctggctgccctttggctctctcctgctgtgcctgttatcttcccctgccacccgccccaaggcttttgcctagttccccagtattctcgctggggattgaataaagcaagacaagacccgtaaaaaaaaaaaaaaaaaaaaaaaaaa

SEQ ID NO: 6 - DNA, 723 bp, Bovine
  source 1..723: mol_type = genomic DNA
agtgcttccggccagctccctgatcctgctagaccatctgtcccaggctccaagctgctccacaggcatcatgcggagcaccctgctgtttgcagtcatcctggccctcagctcagctcggagtttgggtgcggtctgtgaggagtcacaggagcaggtggtgcctggtgggggtcacagcaagaaggactcaaatctctaccagctgcccccatcattgctccggagactctatgatagccgcgtggtctccctggatggattgctcaagatgctgagcaaggccagcgtaggtcctaaggagtcaccacttccccagaaacgtgacatgcatgacttctttgtgggtctcatgggcaagaggaacctccagccagacactcctgttgatataaaccaagaaaacatccccagctttggcaccttcaagtaccctccaagtgtggaatgagcactccactcctggactcctgggctacatcgtgaagacacccacccctggatgcacatgcttctatttcccttcctcctccctacccctgtaacactcttgtgctttgaccccttcttctctctgtcccactggctgcagaaactgccttgtgagcatccccagtccctgtaatcattgactacagatggccctggattttctgtagcatcctacaaatataatgtctctctctattcctcaacaataaaggatttttacatattatgacc

SEQ ID NO: 7 - DNA, 798 bp, Bovine
  source 1..798: mol_type = genomic DNA
atctgcttctctaatcactactcacagtaacctcaactcctgccacaatgtacaagatacaactcttgtcttgcattgcactaactcttgcactcgttgcaaacggtgcacctacttcaagctctacggggaacacaatgaaagaagtgaagtcattgctgctggatttacagttgcttttggagaaagttaaaaatcctgagaacctcaagctctccaggatgcatacatttgacttttacgtgcccaaggttaacgctacagaattgaaacatcttaagtgtttactagaagaactcaaacttctagaggaagtgctaaatttagctccaagcaaaaacctgaaccccagagagatcaaggattcaatggacaatatcaagagaatcgttttggaactacagggatctgaaacaagattcacatgtgaatatgatgatgcaacagtaaacgctgtagaatttctgaacaaatggattaccttttgtcaaagcatctactcaacaatgacttgatcactaagtgcctctcattttaaactatcaggctttctatttatttaaatatttaaaatttatatttattttttgatatatgttttcctaccttttgtaactgttagtcttaagatgataaatatggatcttttaagattctttttgtaagccctacgggctctaaaaaattcagttaaattatttatcctgaagtatttatttgtatattgaatttttaaatataatgtctatgcaggtcattgactaaaattatttaataaagttgatgaataaaaacaaa

SEQ ID NO: 8 - DNA, 1244 bp, Bovine
  source 1..1244: mol_type = genomic DNA
ctccagggactccactgcgtgttccctgctggcttaaggccgggaggccccatcctgcaggcaaaaccgatcctgggaccgacggagggtcagccaccacagcccctgctggactcagaggtctcccagctcctttttctgtgcgctgctcacgacactccaaaaaccttctctaagaagtgcagccactgggagcactgctagctggtagaaccatgctgcagaactccagccacagggaagccatggtccatgtggataagacccggagggagcaggacagggaaggggtgtgggcagcggcagggggagccctggcccccagcacctcctccccattctcccctgagcccccaggggcctcaggcagcatcatccctgtctactgtgccctcctggccaccgtggtccttggtctgcttgcctacgtggtcttcaagtgctggcgctcacgcaaacacaggcagcagctggccaaagctcggaccgcagagctgggggccctcagcagggaccagctccatggggacagcagtgtctttcgggactctccagctggcctggagccctgtgcccccagccaagggccgccgcctgaacttggctgccagctctacctccaccttcctcggcagcagcaggaggaagtggaacggctcctggaggtgtcgggtgaaccggccaacggctggcggggcctggcgggccgcctgggctaccaggctgaggcagtggagaccatggcccggagcccagggcccgcctctgccctgctgagggactgggctgtccaggaaggcagtggcgccaccctcagagcgctagcagacgcccttgctgccatgggccgtgaagacgtgattcgggctctgagctccccggctgagggttgctctgtggtgtgagttgtggctccacagcctggcctctcagggaacctgctctggtgctccccaccacccccacctcatataccttcccctttatgggcttcctggcattggtgacctcagcttgttctgttttggggggacacacaaaacaccagtcacctcccctccccctgccttcttccaggacagggatcaggacgtgggcgggagacagccaggcagggagcagcagtcttgccctgccccaatccccacccacctccccatagtctcaactgttttttctacttttgtaccccatattaaaggcaactctggactgaaaaaaaaaaaaaaaaaaaaaaaaaaaaa

SEQ ID NO: 9 - DNA, 19 bp, synthetic construct
  source 1..19: mol_type = other DNA
aggatcacagcgaggagaa

SEQ ID NO: 10 - DNA, 20 bp, synthetic construct
  source 1..20: mol_type = other DNA
ggcatgttgcatggtctttc

SEQ ID NO: 11 - DNA, 24 bp, synthetic construct
  source 1..24: mol_type = other DNA
aaagtctaccctccgcagcaacat

SEQ ID NO: 12 - DNA, 24 bp, synthetic construct
  source 1..24: mol_type = other DNA
catcgataagatgctaaacaaggc

SEQ ID NO: 13 - DNA, 18 bp, synthetic construct
  source 1..18: mol_type = other DNA
actgaggctgctggagta

SEQ ID NO: 14 - DNA, 27 bp, synthetic construct
  source 1..27: mol_type = other DNA
tgccaactgatcaagagagatggaacg

SEQ ID NO: 15 - DNA, 20 bp, synthetic construct
  source 1..20: mol_type = other DNA
ccgctcccatggttaagaaa

SEQ ID NO: 16 - DNA, 22 bp, synthetic construct
  source 1..22: mol_type = other DNA
gtctacttctggaacagccatc

SEQ ID NO: 17 - DNA, 24 bp, synthetic construct
  source 1..24: mol_type = other DNA
taggccagctctaactgaccaggt

SEQ ID NO: 18 - DNA, 19 bp, synthetic construct
  source 1..19: mol_type = other DNA
agcacaggtgacaacatcc

SEQ ID NO: 19 - DNA, 19 bp, synthetic construct
  source 1..19: mol_type = other DNA
agcacgatcatgcagaaca

SEQ ID NO: 20 - DNA, 24 bp, synthetic construct
  source 1..24: mol_type = other DNA
tcatcgccctgtggaatgtcttca

SEQ ID NO: 21 - DNA, 20 bp, synthetic construct
  source 1..20: mol_type = other DNA
ggaaagttggcaccatctca

SEQ ID NO: 22 - DNA, 22 bp, synthetic construct
  source 1..22: mol_type = other DNA
gtctgaacttgatggcccatag

SEQ ID NO: 23 - DNA, 24 bp, synthetic construct
  source 1..24: mol_type = other DNA
caacagttgcagtttcgctggtcc

SEQ ID NO: 24 - DNA, 21 bp, synthetic construct
  source 1..21: mol_type = other DNA
cctggatggattgctcaagat

SEQ ID NO: 25 - DNA, 20 bp, synthetic construct
  source 1..20: mol_type = other DNA
cccatgagacccacaaagaa

SEQ ID NO: 26 - DNA, 24 bp, synthetic construct
  source 1..24: mol_type = other DNA
agcgtaggtcctaaggagtcacca

SEQ ID NO: 27 - DNA, 21 bp, synthetic construct
  source 1..21: mol_type = other DNA
tgcacctacttcaagctctac

SEQ ID NO: 28 - DNA, 21 bp, synthetic construct
  source 1..21: mol_type = other DNA
agcttgaggttctcaggattt

SEQ ID NO: 29 - DNA, 27 bp, synthetic construct
  source 1..27: mol_type = other DNA
agcaactgtaaatccagcagcaatgac

SEQ ID NO: 30 - DNA, 20 bp, synthetic construct
  source 1..20: mol_type = other DNA
gttgctctgtggtgtgagtt

SEQ ID NO: 31 - DNA, 20 bp, synthetic construct
  source 1..20: mol_type = other DNA
atgccaggaagcccataaag

SEQ ID NO: 32 - DNA, 22 bp, synthetic construct
  source 1..22: mol_type = other DNA
tctcagggaacctgctctggtg

SEQ ID NO: 33 - DNA, 21 bp, synthetic construct
  source 1..21: mol_type = other DNA
cttccagcagatgtggatcag

SEQ ID NO: 34 - DNA, 20 bp, synthetic construct
  source 1..20: mol_type = other DNA
aagggtgtaacgcagctaac

SEQ ID NO: 35 - DNA, 24 bp, synthetic construct
  source 1..24: mol_type = other DNA
tcgtccaccgcaaatgcttctagg